European Patent Application EP 4 183 878 A1, published May 24, 2023. Title: PVA Membrane Immobilized Enzyme and Preparation Method therefor. Applicant: ASYMCHEM LIFE SCIENCE (TIANJIN) CO., LTD. The sequence listing filed with the application follows.

SEQUENCE LISTING (5 sequences)

SEQ ID NO: 1 - protein, 459 aa, Chromobacterium violaceum DSM30191
MQKQRTTSQWRELDAAHHLHPFTDTASLNQAGARVMTRGEGVYLWDSEGNKIIDGMAGLWCVNVGYGRKDFAEAARRQMEELPFYNTFFKTTHPAVVELSSLLAEVTPAGFDRVFYTNSGSESVDTMIRMVRRYWDVQGKPEKKTLIGRWNGYHGSTIGGASLGGMKYMHEQGDLPIPGMAHIEQPWWYKHGKDMTPDEFGVVAARWLEEKILEIGADKVAAFVGEPIQGAGGVIVPPATYWPEIERICRKYDVLLVADEVICGFGRTGEWFGHQHFGFQPDLFTAAKGLSSGYLPIGAVFVGKRVAEGLIAGGDFNHGFTYSGHPVCAAVAHANVAALRDEGIVQRVKDDIGPYMQKRWRETFSRFEHVDDVRGVGMVQAFTLVKNKAKRELFPDFGEIGTLCRDIFFRNNLIMRACGDHIVSAPPLVMTRAEVDEMLAVAERCLEEFEQTLKARGLA

SEQ ID NO: 2 - protein, 476 aa, Arthrobacter citreus
MGLTVQKINWEQVKEWDRKYLMRTFSTQNEYQPVPIESTEGDYLITPGGTRLLDFFNQLCCVNLGQKNQKVNAAIKEALDRYGFVWDTYATDYKAKAAKIIIEDILGDEDWPGKVRFVSTGSEAVETALNIARLYTNRPLVVTREHDYHGWTGGAATVTRLRSFRSGLVGENSESFSAQIPGSSCSSAVLMAPSSNTFQDSNGNYLKDENGELLSVKYTRRMIENYGPEQVAAVITEVSQGVGSTMPPYEYVPQIRKMTKELGVLWISDEVLTGFGRTGKWFGYQHYGVQPDIITMGKGLSSSSLPAGAVVVSKEIAAFMDKHRWESVSTYAGHPVAMAAVCANLEVMMEENLVEQAKNSGEYIRSKLELLQEKHKSIGNFDGYGLLWIVDIVNAKTKTPYVKLDRNFRHGMNPNQIPTQIIMEKALEKGVLIGGAMPNTMRIGASLNVSRGDIDKAMDALDYALDYLESGEWQQS

SEQ ID NO: 3 - protein, 253 aa, Acetobacter sp. CCTCC M209061
MARVAGKVAIVSGAANGIGKATAQLLAKEGAKVVIGDLKEEDGQKAVAEIKAAGGEAAFVKLNVTDEAAWKAAIGQTLKLYGRLDIAVNNAGINYSGSVESTSLEDWRRVQSINLDGVFLGTQVAIEAMKKSGGGSIVNLSSISGLIGDPMLAAYVASKGGVRLFTKSAALHCAKSGYKIRVNSVHPGYIWTPMVAGLTKEDAAARQKLVDLHPIGHLGEPNDIAYGILYLASDESKFVTGSELVIDGGYTAQ

SEQ ID NO: 4 - protein, 541 aa, Rhodococcus sp. Phi1
MTAQISPTVVDAVVIGAGFGGIYAVHKLHNEQGLTVVGFDKADGPGGTWYWNRYPGALSDTESHLYRFSFDRDLLQDGTWKTTYITQPEILEYLESVVDRFDLRRHFRFGTEVTSAIYLEDENLWEVSTDKGEVYRAKYVVNAVGLLSAINFPDLPGLDTFEGETIHTAAWPEGKNLAGKRVGVIGTGSTGQQVITALAPEVEHLTVFVRTPQYSVPVGNRPVTKEQIDAIKADYDGIWDSVKKSAVAFGFEESTLPAMSVSEEERNRIFQEAWDHGGGFRFMFGTFGDIATDEAANEAAASFIRSKIAEIIEDPETARKLMPTGLYAKRPLCDNGYYEVYNRPNVEAVAIKENPIREVTAKGVVTEDGVLHELDVLVFATGFDAVDGNYRRIEIRGRNGLHINDHWDGQPTSYLGVTTANFPNWFMVLGPNGPFTNLPPSIETQVEWISDTVAYAERNEIRAIEPTPEAEEEWTQTCTDIANATLFTRGDSWIFGANVPGKKPSVLFYLGGLGNYRNVLAGVVADSYRGFELKSAVPVTA

SEQ ID NO: 5 - protein, 603 aa, Rhodococcus ruber-SD1
MTTSIDREALRRKYAEERDKRIRPDGNDQYIRLDHVDGWSHDPYMPITPREPKLDHVTFAFIGGGFSGLVTAARLRESGVESVRIIDKAGDFGGVWYWNRYPGAMCDTAAMVYMPLLEETGYMPTEKYAHGPEILEHCQRIGKHYDLYDDALFHTEVTDLVWQEHDQRWRISTNRGDHFTAQFVGMGTGPLHVAQLPGIPGIESFRGKSFHTSRWDYDYTGGDALGAPMDKLADKRVAVIGTGATAVQCVPELAKYCRELYVVQRTPSAVDERGNHPIDEKWFAQIATPGWQKRWLDSFTAIWDGVLTDPSELAIEHEDLVQDGWTALGQRMRAAVGSVPIEQYSPENVQRALEEADDEQMERIRARVDEIVTDPATAAQLKAWFRQMCKRPCFHDDYLPAFNRPNTHLVDTGGKGVERITENGVVVAGVEYEVDCIVYASGFEFLGTGYTDRAGFDPTGRDGVKLSEHWAQGTRTLHGMHTYGFPNLFVLQLMQGAALGSNIPHNFVEAARVVAAIVDHVLSTGTSSVETTKEAEQAWVQLLLDHGRPLGNPECTPGYYNNEGKPAELKDRLNVGYPAGSAAFFRMMDHWLAAGSFDGLTFR